European Patent Specification EP 3 647 415 B1, published December 3, 2025. Title: Novel modified O-succinyl homoserine transferase and a method of producing O-succinyl homoserine using thereof. Applicant: CJ CheilJedang Corporation. The sequence listing filed with the application follows.

SEQUENCE LISTING (98 sequences)

SEQ ID NO: 1 - protein, 377 aa, Corynebacterium glutamicum
  PEPTIDE (1)..(377): metX
MPTLAPSGQLEIQAIGDVSTEAGAIITNAEIAYHRWGEYRVDKEGRSNVVLIEHALTGDSNAADWWADLLGPGKAINTDIYCVICTNVIGGCNGSTGPGSMHPDGNFWGNRFPATSIRDQVNAEKQFLDALGITTVAAVLGGSMGGARTLEWAAMYPETVGAAAVLAVSARASAWQIGIQSAQIKAIENDHHWHEGNYYESGCNPATGLGAARRIAHLTYRGELEIDERFGTKAQKNENPLGPYRKPDQRFAVESYLDYQADKLVQRFDAGSYVLLTDALNRHDIGRDRGGLNKALESIKVPVLVAGVDTDILYPYHQQEHLSRNLGNLLAMAKIVSPVGHDAFLTESRQMDRIVRNFFSLISPDEDNPSTYIEFYI

SEQ ID NO: 2 - DNA, 1134 bp, Corynebacterium glutamicum
  gene (1)..(1134): metX
atgcccaccctcgcgccttcaggtcaacttgaaatccaagcgatcggtgatgtctccaccgaagccggagcaatcattacaaacgctgaaatcgcctatcaccgctggggtgaataccgcgtagataaagaaggacgcagcaatgtcgttctcatcgaacacgccctcactggagattccaacgcagccgattggtgggctgacttgctcggtcccggcaaagccatcaacactgatatttactgcgtgatctgtaccaacgtcatcggtggttgcaacggttccaccggacctggctccatgcatccagatggaaatttctggggtaatcgcttccccgccacgtccattcgtgatcaggtaaacgccgaaaaacaattcctcgacgcactcggcatcaccacggtcgccgcagtacttggtggttccatgggtggtgcccgcaccctagagtgggccgcaatgtacccagaaactgttggcgcagctgctgttcttgcagtttctgcacgcgccagcgcctggcaaatcggcattcaatccgcccaaattaaggcgattgaaaacgaccaccactggcacgaaggcaactactacgaatccggctgcaacccagccaccggactcggcgccgcccgacgcatcgcccacctcacctaccgtggcgaactagaaatcgacgaacgcttcggcaccaaagcccaaaagaacgaaaacccactcggtccctaccgcaagcccgaccagcgcttcgccgtggaatcctacttggactaccaagcagacaagctagtacagcgtttcgacgccggctcctacgtcttgctcaccgacgccctcaaccgccacgacattggtcgcgaccgcggaggcctcaacaaggcactcgaatccatcaaagttccagtccttgtcgcaggcgtagataccgatattttgtacccctaccaccagcaagaacacctctccagaaacctgggaaatctactggcaatggcaaaaatcgtatcccctgtcggccacgatgctttcctcaccgaaagccgccaaatggatcgcatcgtgaggaacttcttcagcctcatctccccagacgaagacaacccttcgacctacatcgagttctacatctaa

SEQ ID NO: 3 - protein, 379 aa, Pseudomonas aeruginosa
MPTVFPDDSVGLVSPQTLHFNEPLELTSGKSLAEYDLVIETYGELNATQSNAVLICHALSGHHHAAGYHSVDERKPGWWDSCIGPGKPIDTRKFFVVALNNLGGCNGSSGPASINPATGKVYGADFPMVTVEDWVHSQARLADRLGIRQWAAVVGGSLGGMQALQWTISYPERVRHCLCIASAPKLSAQNIAFNEVARQAILSDPEFLGGYFQEQGVIPKRGLKLARMVGHITYLSDDAMGAKFGRVLKTEKLNYDLHSVEFQVESYLRYQGEEFSTRFDANTYLLMTKALDYFDPAAAHGDDLVRTLEGVEADFCLMSFTTDWRFSPARSREIVDALIAAKKNVSYLEIDAPQGHDAFLMPIPRYLQAFSGYMNRISV

SEQ ID NO: 4 - DNA, 1140 bp, Pseudomonas aeruginosa
atgcccacagtcttccccgacgactccgtcggtctggtctccccccagacgctgcacttcaacgaaccgctcgagctgaccagcggcaagtccctggccgagtacgacctggtgatcgaaacctacggcgagctgaatgccacgcagagcaacgcggtgctgatctgccacgccctctccggccaccaccacgccgccggctaccacagcgtcgacgagcgcaagccgggctggtgggacagctgcatcggtccgggcaagccgatcgacacccgcaagttcttcgtcgtcgccctcaacaacctcggcggttgcaacggatccagcggccccgccagcatcaatccggcgaccggcaaggtctacggcgcggacttcccgatggttacggtggaagactgggtgcatagccaggcgcgcctggcagaccgcctcggcatccgccagtgggccgcggtggtcggcggcagcctcggcggcatgcaggcgctgcaatggaccatcagctatcccgagcgcgtccgtcactgcctgtgcatcgccagcgcgccgaagctgtcggcgcagaacatcgccttcaacgaagtcgcccggcaggcgattctttccgaccctgagttcctcggcggctacttccaggagcagggcgtgattcccaagcgcggcctcaagctggcgcggatggtcggccatatcacctacctgtccgacgacgccatgggcgccaagttcggccgtgtactgaagaccgagaagctcaactacgacctgcacagcgtcgagttccaggtcgagagttacctgcgctaccagggcgaggagttctccacccgcttcgacgccaatacctacctgctgatgaccaaggcgctggactacttcgaccccgccgccgcccacggcgacgacctggtgcgcaccctggagggcgtcgaggcggacttctgcctgatgtccttcaccaccgactggcgtttctcgccggcccgctcgcgggaaatcgtcgacgccctgatcgcggcgaaaaagaacgtcagctacctggagatcgacgccccgcaaggccacgacgccttcctcatgccgatcccccggtacctgcaagccttcagcggttacatgaaccgcatcagcgtgtga

SEQ ID NO: 5 - DNA, 28 bp, Artificial Sequence
  primer 1
ggatcccctcgttgttcacccagcaacc

SEQ ID NO: 6 - DNA, 30 bp, Artificial Sequence
  primer 2
ggatcccaaagtcacaactacttatgttag

SEQ ID NO: 7 - DNA, 35 bp, Artificial Sequence
  primer 3
acgcgccagcgcctggaacatcggcattcaatccg

SEQ ID NO: 8 - DNA, 35 bp, Artificial Sequence
  primer 4
cggattgaatgccgatgttccaggcgctggcgcgt

SEQ ID NO: 9 - DNA, 33 bp, Artificial Sequence
  primer 5
gtagataccgatattcggtacccctaccaccag

SEQ ID NO: 10 - DNA, 33 bp, Artificial Sequence
  primer 6
ctggtggtaggggtaccgaatatcggtatctac

SEQ ID NO: 11 - DNA, 24 bp, Artificial Sequence
  primer 7
tctagatgcgctgattatctcacc

SEQ ID NO: 12 - DNA, 40 bp, Artificial Sequence
  primer 8
actggtgggtcatggttgcatatgagatcaactcctgtaa

SEQ ID NO: 13 - DNA, 40 bp, Artificial Sequence
  primer 9
ttacaggagttgatctcatatgcaaccatgacccaccagt

SEQ ID NO: 14 - DNA, 24 bp, Artificial Sequence
  primer 10
tctagaccttgaagttcttgactg

SEQ ID NO: 15 - DNA, 24 bp, Artificial Sequence
  primer 11
tctagaagtagcgttgctgtacac

SEQ ID NO: 16 - DNA, 43 bp, Artificial Sequence
  primer 12
atcaatggtctcgatgcccatatggcatttggaggtccttaag

SEQ ID NO: 17 - DNA, 43 bp, Artificial Sequence
  primer 13
cttaaggacctccaaatgccatatgggcatcgagaccattgat

SEQ ID NO: 18 - DNA, 24 bp, Artificial Sequence
  primer 14
tctagatggaaccgttgcaaccac

SEQ ID NO: 19 - protein, 421 aa, Corynebacterium glutamicum
  PEPTIDE (1)..(421): lysC
MALVVQKYGGSSLESAERIRNVAERIVATKKAGNDVVVVCSAMGDTTDELLELAAAVNPVPPAREMDMLLTAGERISNALVAMAIESLGAEAQSFTGSQAGVLTTERHGNARIVDVTPGRVREALDEGKICIVAGFQGVNKETRDVTTLGRGGSDTTAVALAAALNADVCEIYSDVDGVYTADPRIVPNAQKLEKLSFEEMLELAAVGSKILVLRSVEYARAFNVPLRVRSSYSNDPGTLIAGSMEDIPVEEAVLTGVATDKSEAKVTVLGISDKPGEAAKVFRALADAEINIDMVLQNVSSVEDGTTDITFTCPRSDGRRAMEILKKLQVQGNWTNVLYDDQVGKVSLVGAGMKSHPGVTAEFMEALRDVNVNIELISTSEIRISVLIREDDLDAAARALHEQFQLGGEDEAVVYAGTGR

SEQ ID NO: 20 - DNA, 1266 bp, Corynebacterium glutamicum
  gene (1)..(1266): lysC
atggccctggtcgtacagaaatatggcggttcctcgcttgagagtgcggaacgcattagaaacgtcgctgaacggatcgttgccaccaagaaggctggaaatgatgtcgtggttgtctgctccgcaatgggagacaccacggatgaacttctagaacttgcagcggcagtgaatcccgttccgccagctcgtgaaatggatatgctcctgactgctggtgagcgtatttctaacgctctcgtcgccatggctattgagtcccttggcgcagaagcccaatctttcacgggctctcaggctggtgtgctcaccaccgagcgccacggaaacgcacgcattgttgatgtcactccaggtcgtgtgcgtgaagcactcgatgagggcaagatctgcattgttgctggtttccagggtgttaataaagaaacccgcgatgtcaccacgttgggtcgtggtggttctgacaccactgcagttgcgttggcagctgctttgaacgctgatgtgtgtgagatttactcggacgttgacggtgtgtataccgctgacccgcgcatcgttcctaatgcacagaagctggaaaagctcagcttcgaagaaatgctggaacttgctgctgttggctccaagattttggtgctgcgcagtgttgaatacgctcgtgcattcaatgtgccacttcgcgtacgctcgtcttatagtaatgatcccggcactttgattgccggctctatggaggatattcctgtggaagaagcagtccttaccggtgtcgcaaccgacaagtccgaagccaaagtaaccgttctgggtatttccgataagccaggcgaggctgcgaaggttttccgtgcgttggctgatgcagaaatcaacattgacatggttctgcagaacgtctcttctgtagaagacggcaccaccgacatcaccttcacctgccctcgttccgacggccgccgcgcgatggagatcttgaagaagcttcaggttcagggcaactggaccaatgtgctttacgacgaccaggtcggcaaagtctccctcgtgggtgctggcatgaagtctcacccaggtgttaccgcagagttcatggaagctctgcgcgatgtcaacgtgaacatcgaattgatttccacctctgagattcgtatttccgtgctgatccgtgaagatgatctggatgctgctgcacgtgcattgcatgagcagttccagctgggcggcgaagacgaagccgtcgtttatgcaggcaccggacgctaa

SEQ ID NO: 21 - DNA, 29 bp, Artificial Sequence
  primer 15
tcctctagagctgcgcagtgttgaatacg

SEQ ID NO: 22 - DNA, 23 bp, Artificial Sequence
  primer 16
caccgacatcatcttcacctgcc

SEQ ID NO: 23 - DNA, 23 bp, Artificial Sequence
  primer 17
ggcaggtgaagatgatgtcggtg

SEQ ID NO: 24 - DNA, 29 bp, Artificial Sequence
  primer 18
gactctagagttcacctcagagacgatta

SEQ ID NO: 25 - protein, 421 aa, Corynebacterium glutamicum
  PEPTIDE (1)..(421): lysC variant (T311I)
MALVVQKYGGSSLESAERIRNVAERIVATKKAGNDVVVVCSAMGDTTDELLELAAAVNPVPPAREMDMLLTAGERISNALVAMAIESLGAEAQSFTGSQAGVLTTERHGNARIVDVTPGRVREALDEGKICIVAGFQGVNKETRDVTTLGRGGSDTTAVALAAALNADVCEIYSDVDGVYTADPRIVPNAQKLEKLSFEEMLELAAVGSKILVLRSVEYARAFNVPLRVRSSYSNDPGTLIAGSMEDIPVEEAVLTGVATDKSEAKVTVLGISDKPGEAAKVFRALADAEINIDMVLQNVSSVEDGTTDIIFTCPRSDGRRAMEILKKLQVQGNWTNVLYDDQVGKVSLVGAGMKSHPGVTAEFMEALRDVNVNIELISTSEIRISVLIREDDLDAAARALHEQFQLGGEDEAVVYAGTGR

SEQ ID NO: 26 - DNA, 1266 bp, Corynebacterium glutamicum
  gene (1)..(1266): lysC variant (T311I)
atggccctggtcgtacagaaatatggcggttcctcgcttgagagtgcggaacgcattagaaacgtcgctgaacggatcgttgccaccaagaaggctggaaatgatgtcgtggttgtctgctccgcaatgggagacaccacggatgaacttctagaacttgcagcggcagtgaatcccgttccgccagctcgtgaaatggatatgctcctgactgctggtgagcgtatttctaacgctctcgtcgccatggctattgagtcccttggcgcagaagcccaatctttcacgggctctcaggctggtgtgctcaccaccgagcgccacggaaacgcacgcattgttgatgtcactccaggtcgtgtgcgtgaagcactcgatgagggcaagatctgcattgttgctggtttccagggtgttaataaagaaacccgcgatgtcaccacgttgggtcgtggtggttctgacaccactgcagttgcgttggcagctgctttgaacgctgatgtgtgtgagatttactcggacgttgacggtgtgtataccgctgacccgcgcatcgttcctaatgcacagaagctggaaaagctcagcttcgaagaaatgctggaacttgctgctgttggctccaagattttggtgctgcgcagtgttgaatacgctcgtgcattcaatgtgccacttcgcgtacgctcgtcttatagtaatgatcccggcactttgattgccggctctatggaggatattcctgtggaagaagcagtccttaccggtgtcgcaaccgacaagtccgaagccaaagtaaccgttctgggtatttccgataagccaggcgaggctgcgaaggttttccgtgcgttggctgatgcagaaatcaacattgacatggttctgcagaacgtctcttctgtagaagacggcaccaccgacatcatcttcacctgccctcgttccgacggccgccgcgcgatggagatcttgaagaagcttcaggttcagggcaactggaccaatgtgctttacgacgaccaggtcggcaaagtctccctcgtgggtgctggcatgaagtctcacccaggtgttaccgcagagttcatggaagctctgcgcgatgtcaacgtgaacatcgaattgatttccacctctgagattcgtatttccgtgctgatccgtgaagatgatctggatgctgctgcacgtgcattgcatgagcagttccagctgggcggcgaagacgaagccgtcgtttatgcaggcaccggacgctaa

SEQ ID NO: 27 - DNA, 35 bp, Artificial Sequence
  Forward primer for Q176F,L313R
acgcgccagcgcctggtttatcggcattcaatccg

SEQ ID NO: 28 - DNA, 35 bp, Artificial Sequence
  Reverse primer for Q176F,L313R
cggattgaatgccgataaaccaggcgctggcgcgt

SEQ ID NO: 29 - DNA, 35 bp, Artificial Sequence
  Forward primer for Q176S,L313R
acgcgccagcgcctggtctatcggcattcaatccg

SEQ ID NO: 30 - DNA, 35 bp, Artificial Sequence
  Reverse primer for Q176S,L313R
cggattgaatgccgatagaccaggcgctggcgcgt

SEQ ID NO: 31 - DNA, 35 bp, Artificial Sequence
  Forward primer for Q176Y,L313R
acgcgccagcgcctggtatatcggcattcaatccg

SEQ ID NO: 32 - DNA, 35 bp, Artificial Sequence
  Reverse primer for Q176Y,L313R
cggattgaatgccgatataccaggcgctggcgcgt

SEQ ID NO: 33 - DNA, 35 bp, Artificial Sequence
  Forward primer for Q176C,L313R
acgcgccagcgcctggtgcatcggcattcaatccg

SEQ ID NO: 34 - DNA, 35 bp, Artificial Sequence
  Reverse primer for Q176C,L313R
cggattgaatgccgatgcaccaggcgctggcgcgt

SEQ ID NO: 35 - DNA, 35 bp, Artificial Sequence
  Forward primer for Q176P,L313R
acgcgccagcgcctggccaatcggcattcaatccg

SEQ ID NO: 36 - DNA, 35 bp, Artificial Sequence
  Reverse primer for Q176P,L313R
cggattgaatgccgattggccaggcgctggcgcgt

SEQ ID NO: 37 - DNA, 35 bp, Artificial Sequence
  Forward primer for Q176H,L313R
acgcgccagcgcctggcacatcggcattcaatccg

SEQ ID NO: 38 - DNA, 35 bp, Artificial Sequence
  Reverse primer for Q176H,L313R
cggattgaatgccgatgtgccaggcgctggcgcgt

SEQ ID NO: 39 - DNA, 35 bp, Artificial Sequence
  Forward primer for Q176L,L313R
acgcgccagcgcctggctcatcggcattcaatccg

SEQ ID NO: 40 - DNA, 35 bp, Artificial Sequence
  Reverse primer for Q176L,L313R
cggattgaatgccgatgagccaggcgctggcgcgt

SEQ ID NO: 41 - DNA, 35 bp, Artificial Sequence
  Forward primer for Q176I,L313R
acgcgccagcgcctggattatcggcattcaatccg

SEQ ID NO: 42 - DNA, 35 bp, Artificial Sequence
  Reverse primer for Q176I,L313R
cggattgaatgccgataatccaggcgctggcgcgt

SEQ ID NO: 43 - DNA, 35 bp, Artificial Sequence
  Forward primer for Q176T,L313R
acgcgccagcgcctggactatcggcattcaatccg

SEQ ID NO: 44 - DNA, 35 bp, Artificial Sequence
  Reverse primer for Q176T,L313R
cggattgaatgccgatagtccaggcgctggcgcgt

SEQ ID NO: 45 - DNA, 35 bp, Artificial Sequence
  Forward primer for Q176R,L313R
acgcgccagcgcctggcgcatcggcattcaatccg

SEQ ID NO: 46 - DNA, 35 bp, Artificial Sequence
  Reverse primer for Q176R,L313R
cggattgaatgccgatgcgccaggcgctggcgcgt

SEQ ID NO: 47 - DNA, 35 bp, Artificial Sequence
  Forward primer for Q176K,L313R
acgcgccagcgcctggaaaatcggcattcaatccg

SEQ ID NO: 48 - DNA, 35 bp, Artificial Sequence
  Reverse primer for Q176K,L313R
cggattgaatgccgattttccaggcgctggcgcgt

SEQ ID NO: 49 - DNA, 35 bp, Artificial Sequence
  Forward primer for Q176V,L313R
acgcgccagcgcctgggttatcggcattcaatccg

SEQ ID NO: 50 - DNA, 35 bp, Artificial Sequence
  Reverse primer for Q176V,L313R
cggattgaatgccgataacccaggcgctggcgcgt

SEQ ID NO: 51 - DNA, 35 bp, Artificial Sequence
  Forward primer for Q176A,L313R
acgcgccagcgcctgggcaatcggcattcaatccg

SEQ ID NO: 52 - DNA, 35 bp, Artificial Sequence
  Reverse primer for Q176A,L313R
cggattgaatgccgattgcccaggcgctggcgcgt

SEQ ID NO: 53 - DNA, 35 bp, Artificial Sequence
  Forward primer for Q176D,L313R
acgcgccagcgcctgggacatcggcattcaatccg

SEQ ID NO: 54 - DNA, 35 bp, Artificial Sequence
  Reverse primer for Q176D,L313R
cggattgaatgccgatgtcccaggcgctggcgcgt

SEQ ID NO: 55 - DNA, 35 bp, Artificial Sequence
  Forward primer for Q176E,L313R
acgcgccagcgcctgggagatcggcattcaatccg

SEQ ID NO: 56 - DNA, 35 bp, Artificial Sequence
  Reverse primer for Q176E,L313R
cggattgaatgccgatctcccaggcgctggcgcgt

SEQ ID NO: 57 - DNA, 35 bp, Artificial Sequence
  Forward primer for Q176G,L313R
acgcgccagcgcctggggcatcggcattcaatccg

SEQ ID NO: 58 - DNA, 35 bp, Artificial Sequence
  Reverse primer for Q176G,L313R
cggattgaatgccgatgccccaggcgctggcgcgt

SEQ ID NO: 59 - DNA, 35 bp, Artificial Sequence
  Forward primer for Q176W,L313R
acgcgccagcgcctggtggatcggcattcaatccg

SEQ ID NO: 60 - DNA, 35 bp, Artificial Sequence
  Reverse primer for Q176W,L313R
cggattgaatgccgatccaccaggcgctggcgcgt

SEQ ID NO: 61 - protein, 377 aa, Artificial Sequence
  metX L313R
MPTLAPSGQLEIQAIGDVSTEAGAIITNAEIAYHRWGEYRVDKEGRSNVVLIEHALTGDSNAADWWADLLGPGKAINTDIYCVICTNVIGGCNGSTGPGSMHPDGNFWGNRFPATSIRDQVNAEKQFLDALGITTVAAVLGGSMGGARTLEWAAMYPETVGAAAVLAVSARASAWQIGIQSAQIKAIENDHHWHEGNYYESGCNPATGLGAARRIAHLTYRGELEIDERFGTKAQKNENPLGPYRKPDQRFAVESYLDYQADKLVQRFDAGSYVLLTDALNRHDIGRDRGGLNKALESIKVPVLVAGVDTDIRYPYHQQEHLSRNLGNLLAMAKIVSPVGHDAFLTESRQMDRIVRNFFSLISPDEDNPSTYIEFYI

SEQ ID NO: 62 - DNA, 1134 bp, Artificial Sequence
  metX L313R
atgcccaccctcgcgccttcaggtcaacttgaaatccaagcgatcggtgatgtctccaccgaagccggagcaatcattacaaacgctgaaatcgcctatcaccgctggggtgaataccgcgtagataaagaaggacgcagcaatgtcgttctcatcgaacacgccctcactggagattccaacgcagccgattggtgggctgacttgctcggtcccggcaaagccatcaacactgatatttactgcgtgatctgtaccaacgtcatcggtggttgcaacggttccaccggacctggctccatgcatccagatggaaatttctggggtaatcgcttccccgccacgtccattcgtgatcaggtaaacgccgaaaaacaattcctcgacgcactcggcatcaccacggtcgccgcagtacttggtggttccatgggtggtgcccgcaccctagagtgggccgcaatgtacccagaaactgttggcgcagctgctgttcttgcagtttctgcacgcgccagcgcctggcaaatcggcattcaatccgcccaaattaaggcgattgaaaacgaccaccactggcacgaaggcaactactacgaatccggctgcaacccagccaccggactcggcgccgcccgacgcatcgcccacctcacctaccgtggcgaactagaaatcgacgaacgcttcggcaccaaagcccaaaagaacgaaaacccactcggtccctaccgcaagcccgaccagcgcttcgccgtggaatcctacttggactaccaagcagacaagctagtacagcgtttcgacgccggctcctacgtcttgctcaccgacgccctcaaccgccacgacattggtcgcgaccgcggaggcctcaacaaggcactcgaatccatcaaagttccagtccttgtcgcaggcgtagataccgatattcggtacccctaccaccagcaagaacacctctccagaaacctgggaaatctactggcaatggcaaaaatcgtatcccctgtcggccacgatgctttcctcaccgaaagccgccaaatggatcgcatcgtgaggaacttcttcagcctcatctccccagacgaagacaacccttcgacctacatcgagttctacatctaa

SEQ ID NO: 63 - protein, 377 aa, Artificial Sequence
  metX Q176N_L313R
MPTLAPSGQLEIQAIGDVSTEAGAIITNAEIAYHRWGEYRVDKEGRSNVVLIEHALTGDSNAADWWADLLGPGKAINTDIYCVICTNVIGGCNGSTGPGSMHPDGNFWGNRFPATSIRDQVNAEKQFLDALGITTVAAVLGGSMGGARTLEWAAMYPETVGAAAVLAVSARASAWNIGIQSAQIKAIENDHHWHEGNYYESGCNPATGLGAARRIAHLTYRGELEIDERFGTKAQKNENPLGPYRKPDQRFAVESYLDYQADKLVQRFDAGSYVLLTDALNRHDIGRDRGGLNKALESIKVPVLVAGVDTDIRYPYHQQEHLSRNLGNLLAMAKIVSPVGHDAFLTESRQMDRIVRNFFSLISPDEDNPSTYIEFYI

SEQ ID NO: 64 - DNA, 1134 bp, Artificial Sequence
  metX Q176N_L313R
atgcccaccctcgcgccttcaggtcaacttgaaatccaagcgatcggtgatgtctccaccgaagccggagcaatcattacaaacgctgaaatcgcctatcaccgctggggtgaataccgcgtagataaagaaggacgcagcaatgtcgttctcatcgaacacgccctcactggagattccaacgcagccgattggtgggctgacttgctcggtcccggcaaagccatcaacactgatatttactgcgtgatctgtaccaacgtcatcggtggttgcaacggttccaccggacctggctccatgcatccagatggaaatttctggggtaatcgcttccccgccacgtccattcgtgatcaggtaaacgccgaaaaacaattcctcgacgcactcggcatcaccacggtcgccgcagtacttggtggttccatgggtggtgcccgcaccctagagtgggccgcaatgtacccagaaactgttggcgcagctgctgttcttgcagtttctgcacgcgccagcgcctggaacatcggcattcaatccgcccaaattaaggcgattgaaaacgaccaccactggcacgaaggcaactactacgaatccggctgcaacccagccaccggactcggcgccgcccgacgcatcgcccacctcacctaccgtggcgaactagaaatcgacgaacgcttcggcaccaaagcccaaaagaacgaaaacccactcggtccctaccgcaagcccgaccagcgcttcgccgtggaatcctacttggactaccaagcagacaagctagtacagcgtttcgacgccggctcctacgtcttgctcaccgacgccctcaaccgccacgacattggtcgcgaccgcggaggcctcaacaaggcactcgaatccatcaaagttccagtccttgtcgcaggcgtagataccgatattcggtacccctaccaccagcaagaacacctctccagaaacctgggaaatctactggcaatggcaaaaatcgtatcccctgtcggccacgatgctttcctcaccgaaagccgccaaatggatcgcatcgtgaggaacttcttcagcctcatctccccagacgaagacaacccttcgacctacatcgagttctacatctaa

SEQ ID NO: 65 - protein, 377 aa, Artificial Sequence
  Q176F,L313R
MPTLAPSGQLEIQAIGDVSTEAGAIITNAEIAYHRWGEYRVDKEGRSNVVLIEHALTGDSNAADWWADLLGPGKAINTDIYCVICTNVIGGCNGSTGPGSMHPDGNFWGNRFPATSIRDQVNAEKQFLDALGITTVAAVLGGSMGGARTLEWAAMYPETVGAAAVLAVSARASAWFIGIQSAQIKAIENDHHWHEGNYYESGCNPATGLGAARRIAHLTYRGELEIDERFGTKAQKNENPLGPYRKPDQRFAVESYLDYQADKLVQRFDAGSYVLLTDALNRHDIGRDRGGLNKALESIKVPVLVAGVDTDIRYPYHQQEHLSRNLGNLLAMAKIVSPVGHDAFLTESRQMDRIVRNFFSLISPDEDNPSTYIEFYI

SEQ ID NO: 66 - DNA, 1134 bp, Artificial Sequence
  Q176F,L313R
atgcccaccctcgcgccttcaggtcaacttgaaatccaagcgatcggtgatgtctccaccgaagccggagcaatcattacaaacgctgaaatcgcctatcaccgctggggtgaataccgcgtagataaagaaggacgcagcaatgtcgttctcatcgaacacgccctcactggagattccaacgcagccgattggtgggctgacttgctcggtcccggcaaagccatcaacactgatatttactgcgtgatctgtaccaacgtcatcggtggttgcaacggttccaccggacctggctccatgcatccagatggaaatttctggggtaatcgcttccccgccacgtccattcgtgatcaggtaaacgccgaaaaacaattcctcgacgcactcggcatcaccacggtcgccgcagtacttggtggttccatgggtggtgcccgcaccctagagtgggccgcaatgtacccagaaactgttggcgcagctgctgttcttgcagtttctgcacgcgccagcgcctggtttatcggcattcaatccgcccaaattaaggcgattgaaaacgaccaccactggcacgaaggcaactactacgaatccggctgcaacccagccaccggactcggcgccgcccgacgcatcgcccacctcacctaccgtggcgaactagaaatcgacgaacgcttcggcaccaaagcccaaaagaacgaaaacccactcggtccctaccgcaagcccgaccagcgcttcgccgtggaatcctacttggactaccaagcagacaagctagtacagcgtttcgacgccggctcctacgtcttgctcaccgacgccctcaaccgccacgacattggtcgcgaccgcggaggcctcaacaaggcactcgaatccatcaaagttccagtccttgtcgcaggcgtagataccgatattcggtacccctaccaccagcaagaacacctctccagaaacctgggaaatctactggcaatggcaaaaatcgtatcccctgtcggccacgatgctttcctcaccgaaagccgccaaatggatcgcatcgtgaggaacttcttcagcctcatctccccagacgaagacaacccttcgacctacatcgagttctacatctaa

SEQ ID NO: 67 - protein, 377 aa, Artificial Sequence
  Q176S,L313R
MPTLAPSGQLEIQAIGDVSTEAGAIITNAEIAYHRWGEYRVDKEGRSNVVLIEHALTGDSNAADWWADLLGPGKAINTDIYCVICTNVIGGCNGSTGPGSMHPDGNFWGNRFPATSIRDQVNAEKQFLDALGITTVAAVLGGSMGGARTLEWAAMYPETVGAAAVLAVSARASAWSIGIQSAQIKAIENDHHWHEGNYYESGCNPATGLGAARRIAHLTYRGELEIDERFGTKAQKNENPLGPYRKPDQRFAVESYLDYQADKLVQRFDAGSYVLLTDALNRHDIGRDRGGLNKALESIKVPVLVAGVDTDIRYPYHQQEHLSRNLGNLLAMAKIVSPVGHDAFLTESRQMDRIVRNFFSLISPDEDNPSTYIEFYI

SEQ ID NO: 68 - DNA, 1134 bp, Artificial Sequence
  Q176S,L313R
atgcccaccctcgcgccttcaggtcaacttgaaatccaagcgatcggtgatgtctccaccgaagccggagcaatcattacaaacgctgaaatcgcctatcaccgctggggtgaataccgcgtagataaagaaggacgcagcaatgtcgttctcatcgaacacgccctcactggagattccaacgcagccgattggtgggctgacttgctcggtcccggcaaagccatcaacactgatatttactgcgtgatctgtaccaacgtcatcggtggttgcaacggttccaccggacctggctccatgcatccagatggaaatttctggggtaatcgcttccccgccacgtccattcgtgatcaggtaaacgccgaaaaacaattcctcgacgcactcggcatcaccacggtcgccgcagtacttggtggttccatgggtggtgcccgcaccctagagtgggccgcaatgtacccagaaactgttggcgcagctgctgttcttgcagtttctgcacgcgccagcgcctggtctatcggcattcaatccgcccaaattaaggcgattgaaaacgaccaccactggcacgaaggcaactactacgaatccggctgcaacccagccaccggactcggcgccgcccgacgcatcgcccacctcacctaccgtggcgaactagaaatcgacgaacgcttcggcaccaaagcccaaaagaacgaaaacccactcggtccctaccgcaagcccgaccagcgcttcgccgtggaatcctacttggactaccaagcagacaagctagtacagcgtttcgacgccggctcctacgtcttgctcaccgacgccctcaaccgccacgacattggtcgcgaccgcggaggcctcaacaaggcactcgaatccatcaaagttccagtccttgtcgcaggcgtagataccgatattcggtacccctaccaccagcaagaacacctctccagaaacctgggaaatctactggcaatggcaaaaatcgtatcccctgtcggccacgatgctttcctcaccgaaagccgccaaatggatcgcatcgtgaggaacttcttcagcctcatctccccagacgaagacaacccttcgacctacatcgagttctacatctaa

SEQ ID NO: 69 - protein, 377 aa, Artificial Sequence
  Q176Y,L313R
MPTLAPSGQLEIQAIGDVSTEAGAIITNAEIAYHRWGEYRVDKEGRSNVVLIEHALTGDSNAADWWADLLGPGKAINTDIYCVICTNVIGGCNGSTGPGSMHPDGNFWGNRFPATSIRDQVNAEKQFLDALGITTVAAVLGGSMGGARTLEWAAMYPETVGAAAVLAVSARASAWYIGIQSAQIKAIENDHHWHEGNYYESGCNPATGLGAARRIAHLTYRGELEIDERFGTKAQKNENPLGPYRKPDQRFAVESYLDYQADKLVQRFDAGSYVLLTDALNRHDIGRDRGGLNKALESIKVPVLVAGVDTDIRYPYHQQEHLSRNLGNLLAMAKIVSPVGHDAFLTESRQMDRIVRNFFSLISPDEDNPSTYIEFYI

SEQ ID NO: 70 - DNA, 1134 bp, Artificial Sequence
  Q176Y,L313R
atgcccaccctcgcgccttcaggtcaacttgaaatccaagcgatcggtgatgtctccaccgaagccggagcaatcattacaaacgctgaaatcgcctatcaccgctggggtgaataccgcgtagataaagaaggacgcagcaatgtcgttctcatcgaacacgccctcactggagattccaacgcagccgattggtgggctgacttgctcggtcccggcaaagccatcaacactgatatttactgcgtgatctgtaccaacgtcatcggtggttgcaacggttccaccggacctggctccatgcatccagatggaaatttctggggtaatcgcttccccgccacgtccattcgtgatcaggtaaacgccgaaaaacaattcctcgacgcactcggcatcaccacggtcgccgcagtacttggtggttccatgggtggtgcccgcaccctagagtgggccgcaatgtacccagaaactgttggcgcagctgctgttcttgcagtttctgcacgcgccagcgcctggtatatcggcattcaatccgcccaaattaaggcgattgaaaacgaccaccactggcacgaaggcaactactacgaatccggctgcaacccagccaccggactcggcgccgcccgacgcatcgcccacctcacctaccgtggcgaactagaaatcgacgaacgcttcggcaccaaagcccaaaagaacgaaaacccactcggtccctaccgcaagcccgaccagcgcttcgccgtggaatcctacttggactaccaagcagacaagctagtacagcgtttcgacgccggctcctacgtcttgctcaccgacgccctcaaccgccacgacattggtcgcgaccgcggaggcctcaacaaggcactcgaatccatcaaagttccagtccttgtcgcaggcgtagataccgatattcggtacccctaccaccagcaagaacacctctccagaaacctgggaaatctactggcaatggcaaaaatcgtatcccctgtcggccacgatgctttcctcaccgaaagccgccaaatggatcgcatcgtgaggaacttcttcagcctcatctccccagacgaagacaacccttcgacctacatcgagttctacatctaa

SEQ ID NO: 71 - protein, 377 aa, Artificial Sequence
  Q176C,L313R
MPTLAPSGQLEIQAIGDVSTEAGAIITNAEIAYHRWGEYRVDKEGRSNVVLIEHALTGDSNAADWWADLLGPGKAINTDIYCVICTNVIGGCNGSTGPGSMHPDGNFWGNRFPATSIRDQVNAEKQFLDALGITTVAAVLGGSMGGARTLEWAAMYPETVGAAAVLAVSARASAWCIGIQSAQIKAIENDHHWHEGNYYESGCNPATGLGAARRIAHLTYRGELEIDERFGTKAQKNENPLGPYRKPDQRFAVESYLDYQADKLVQRFDAGSYVLLTDALNRHDIGRDRGGLNKALESIKVPVLVAGVDTDIRYPYHQQEHLSRNLGNLLAMAKIVSPVGHDAFLTESRQMDRIVRNFFSLISPDEDNPSTYIEFYI

SEQ ID NO: 72 - DNA, 1134 bp, Artificial Sequence
  Q176C,L313R
atgcccaccctcgcgccttcaggtcaacttgaaatccaagcgatcggtgatgtctccaccgaagccggagcaatcattacaaacgctgaaatcgcctatcaccgctggggtgaataccgcgtagataaagaaggacgcagcaatgtcgttctcatcgaacacgccctcactggagattccaacgcagccgattggtgggctgacttgctcggtcccggcaaagccatcaacactgatatttactgcgtgatctgtaccaacgtcatcggtggttgcaacggttccaccggacctggctccatgcatccagatggaaatttctggggtaatcgcttccccgccacgtccattcgtgatcaggtaaacgccgaaaaacaattcctcgacgcactcggcatcaccacggtcgccgcagtacttggtggttccatgggtggtgcccgcaccctagagtgggccgcaatgtacccagaaactgttggcgcagctgctgttcttgcagtttctgcacgcgccagcgcctggtgtatcggcattcaatccgcccaaattaaggcgattgaaaacgaccaccactggcacgaaggcaactactacgaatccggctgcaacccagccaccggactcggcgccgcccgacgcatcgcccacctcacctaccgtggcgaactagaaatcgacgaacgcttcggcaccaaagcccaaaagaacgaaaacccactcggtccctaccgcaagcccgaccagcgcttcgccgtggaatcctacttggactaccaagcagacaagctagtacagcgtttcgacgccggctcctacgtcttgctcaccgacgccctcaaccgccacgacattggtcgcgaccgcggaggcctcaacaaggcactcgaatccatcaaagttccagtccttgtcgcaggcgtagataccgatattcggtacccctaccaccagcaagaacacctctccagaaacctgggaaatctactggcaatggcaaaaatcgtatcccctgtcggccacgatgctttcctcaccgaaagccgccaaatggatcgcatcgtgaggaacttcttcagcctcatctccccagacgaagacaacccttcgacctacatcgagttctacatctaa

SEQ ID NO: 73 - protein, 377 aa, Artificial Sequence
  Q176P,L313R
MPTLAPSGQLEIQAIGDVSTEAGAIITNAEIAYHRWGEYRVDKEGRSNVVLIEHALTGDSNAADWWADLLGPGKAINTDIYCVICTNVIGGCNGSTGPGSMHPDGNFWGNRFPATSIRDQVNAEKQFLDALGITTVAAVLGGSMGGARTLEWAAMYPETVGAAAVLAVSARASAWPIGIQSAQIKAIENDHHWHEGNYYESGCNPATGLGAARRIAHLTYRGELEIDERFGTKAQKNENPLGPYRKPDQRFAVESYLDYQADKLVQRFDAGSYVLLTDALNRHDIGRDRGGLNKALESIKVPVLVAGVDTDIRYPYHQQEHLSRNLGNLLAMAKIVSPVGHDAFLTESRQMDRIVRNFFSLISPDEDNPSTYIEFYI

SEQ ID NO: 74 - DNA, 1134 bp, Artificial Sequence
  Q176P,L313R
atgcccaccctcgcgccttcaggtcaacttgaaatccaagcgatcggtgatgtctccaccgaagccggagcaatcattacaaacgctgaaatcgcctatcaccgctggggtgaataccgcgtagataaagaaggacgcagcaatgtcgttctcatcgaacacgccctcactggagattccaacgcagccgattggtgggctgacttgctcggtcccggcaaagccatcaacactgatatttactgcgtgatctgtaccaacgtcatcggtggttgcaacggttccaccggacctggctccatgcatccagatggaaatttctggggtaatcgcttccccgccacgtccattcgtgatcaggtaaacgccgaaaaacaattcctcgacgcactcggcatcaccacggtcgccgcagtacttggtggttccatgggtggtgcccgcaccctagagtgggccgcaatgtacccagaaactgttggcgcagctgctgttcttgcagtttctgcacgcgccagcgcctggccaatcggcattcaatccgcccaaattaaggcgattgaaaacgaccaccactggcacgaaggcaactactacgaatccggctgcaacccagccaccggactcggcgccgcccgacgcatcgcccacctcacctaccgtggcgaactagaaatcgacgaacgcttcggcaccaaagcccaaaagaacgaaaacccactcggtccctaccgcaagcccgaccagcgcttcgccgtggaatcctacttggactaccaagcagacaagctagtacagcgtttcgacgccggctcctacgtcttgctcaccgacgccctcaaccgccacgacattggtcgcgaccgcggaggcctcaacaaggcactcgaatccatcaaagttccagtccttgtcgcaggcgtagataccgatattcggtacccctaccaccagcaagaacacctctccagaaacctgggaaatctactggcaatggcaaaaatcgtatcccctgtcggccacgatgctttcctcaccgaaagccgccaaatggatcgcatcgtgaggaacttcttcagcctcatctccccagacgaagacaacccttcgacctacatcgagttctacatctaa

SEQ ID NO: 75 - protein, 377 aa, Artificial Sequence
  Q176H,L313R
MPTLAPSGQLEIQAIGDVSTEAGAIITNAEIAYHRWGEYRVDKEGRSNVVLIEHALTGDSNAADWWADLLGPGKAINTDIYCVICTNVIGGCNGSTGPGSMHPDGNFWGNRFPATSIRDQVNAEKQFLDALGITTVAAVLGGSMGGARTLEWAAMYPETVGAAAVLAVSARASAWHIGIQSAQIKAIENDHHWHEGNYYESGCNPATGLGAARRIAHLTYRGELEIDERFGTKAQKNENPLGPYRKPDQRFAVESYLDYQADKLVQRFDAGSYVLLTDALNRHDIGRDRGGLNKALESIKVPVLVAGVDTDIRYPYHQQEHLSRNLGNLLAMAKIVSPVGHDAFLTESRQMDRIVRNFFSLISPDEDNPSTYIEFYI

SEQ ID NO: 76 - DNA, 1134 bp, Artificial Sequence
  Q176H,L313R
atgcccaccctcgcgccttcaggtcaacttgaaatccaagcgatcggtgatgtctccaccgaagccggagcaatcattacaaacgctgaaatcgcctatcaccgctggggtgaataccgcgtagataaagaaggacgcagcaatgtcgttctcatcgaacacgccctcactggagattccaacgcagccgattggtgggctgacttgctcggtcccggcaaagccatcaacactgatatttactgcgtgatctgtaccaacgtcatcggtggttgcaacggttccaccggacctggctccatgcatccagatggaaatttctggggtaatcgcttccccgccacgtccattcgtgatcaggtaaacgccgaaaaacaattcctcgacgcactcggcatcaccacggtcgccgcagtacttggtggttccatgggtggtgcccgcaccctagagtgggccgcaatgtacccagaaactgttggcgcagctgctgttcttgcagtttctgcacgcgccagcgcctggcacatcggcattcaatccgcccaaattaaggcgattgaaaacgaccaccactggcacgaaggcaactactacgaatccggctgcaacccagccaccggactcggcgccgcccgacgcatcgcccacctcacctaccgtggcgaactagaaatcgacgaacgcttcggcaccaaagcccaaaagaacgaaaacccactcggtccctaccgcaagcccgaccagcgcttcgccgtggaatcctacttggactaccaagcagacaagctagtacagcgtttcgacgccggctcctacgtcttgctcaccgacgccctcaaccgccacgacattggtcgcgaccgcggaggcctcaacaaggcactcgaatccatcaaagttccagtccttgtcgcaggcgtagataccgatattcggtacccctaccaccagcaagaacacctctccagaaacctgggaaatctactggcaatggcaaaaatcgtatcccctgtcggccacgatgctttcctcaccgaaagccgccaaatggatcgcatcgtgaggaacttcttcagcctcatctccccagacgaagacaacccttcgacctacatcgagttctacatctaa

SEQ ID NO: 77 - protein, 377 aa, Artificial Sequence
  Q176L,L313R
MPTLAPSGQLEIQAIGDVSTEAGAIITNAEIAYHRWGEYRVDKEGRSNVVLIEHALTGDSNAADWWADLLGPGKAINTDIYCVICTNVIGGCNGSTGPGSMHPDGNFWGNRFPATSIRDQVNAEKQFLDALGITTVAAVLGGSMGGARTLEWAAMYPETVGAAAVLAVSARASAWLIGIQSAQIKAIENDHHWHEGNYYESGCNPATGLGAARRIAHLTYRGELEIDERFGTKAQKNENPLGPYRKPDQRFAVESYLDYQADKLVQRFDAGSYVLLTDALNRHDIGRDRGGLNKALESIKVPVLVAGVDTDIRYPYHQQEHLSRNLGNLLAMAKIVSPVGHDAFLTESRQMDRIVRNFFSLISPDEDNPSTYIEFYI

SEQ ID NO: 78 - DNA, 1134 bp, Artificial Sequence
  Q176L,L313R
atgcccaccctcgcgccttcaggtcaacttgaaatccaagcgatcggtgatgtctccaccgaagccggagcaatcattacaaacgctgaaatcgcctatcaccgctggggtgaataccgcgtagataaagaaggacgcagcaatgtcgttctcatcgaacacgccctcactggagattccaacgcagccgattggtgggctgacttgctcggtcccggcaaagccatcaacactgatatttactgcgtgatctgtaccaacgtcatcggtggttgcaacggttccaccggacctggctccatgcatccagatggaaatttctggggtaatcgcttccccgccacgtccattcgtgatcaggtaaacgccgaaaaacaattcctcgacgcactcggcatcaccacggtcgccgcagtacttggtggttccatgggtggtgcccgcaccctagagtgggccgcaatgtacccagaaactgttggcgcagctgctgttcttgcagtttctgcacgcgccagcgcctggctcatcggcattcaatccgcccaaattaaggcgattgaaaacgaccaccactggcacgaaggcaactactacgaatccggctgcaacccagccaccggactcggcgccgcccgacgcatcgcccacctcacctaccgtggcgaactagaaatcgacgaacgcttcggcaccaaagcccaaaagaacgaaaacccactcggtccctaccgcaagcccgaccagcgcttcgccgtggaatcctacttggactaccaagcagacaagctagtacagcgtttcgacgccggctcctacgtcttgctcaccgacgccctcaaccgccacgacattggtcgcgaccgcggaggcctcaacaaggcactcgaatccatcaaagttccagtccttgtcgcaggcgtagataccgatattcggtacccctaccaccagcaagaacacctctccagaaacctgggaaatctactggcaatggcaaaaatcgtatcccctgtcggccacgatgctttcctcaccgaaagccgccaaatggatcgcatcgtgaggaacttcttcagcctcatctccccagacgaagacaacccttcgacctacatcgagttctacatctaa

SEQ ID NO: 79 - protein, 377 aa, Artificial Sequence
  Q176I,L313R
MPTLAPSGQLEIQAIGDVSTEAGAIITNAEIAYHRWGEYRVDKEGRSNVVLIEHALTGDSNAADWWADLLGPGKAINTDIYCVICTNVIGGCNGSTGPGSMHPDGNFWGNRFPATSIRDQVNAEKQFLDALGITTVAAVLGGSMGGARTLEWAAMYPETVGAAAVLAVSARASAWIIGIQSAQIKAIENDHHWHEGNYYESGCNPATGLGAARRIAHLTYRGELEIDERFGTKAQKNENPLGPYRKPDQRFAVESYLDYQADKLVQRFDAGSYVLLTDALNRHDIGRDRGGLNKALESIKVPVLVAGVDTDIRYPYHQQEHLSRNLGNLLAMAKIVSPVGHDAFLTESRQMDRIVRNFFSLISPDEDNPSTYIEFYI

SEQ ID NO: 80 - DNA, 1134 bp, Artificial Sequence
  Q176I,L313R
atgcccaccctcgcgccttcaggtcaacttgaaatccaagcgatcggtgatgtctccaccgaagccggagcaatcattacaaacgctgaaatcgcctatcaccgctggggtgaataccgcgtagataaagaaggacgcagcaatgtcgttctcatcgaacacgccctcactggagattccaacgcagccgattggtgggctgacttgctcggtcccggcaaagccatcaacactgatatttactgcgtgatctgtaccaacgtcatcggtggttgcaacggttccaccggacctggctccatgcatccagatggaaatttctggggtaatcgcttccccgccacgtccattcgtgatcaggtaaacgccgaaaaacaattcctcgacgcactcggcatcaccacggtcgccgcagtacttggtggttccatgggtggtgcccgcaccctagagtgggccgcaatgtacccagaaactgttggcgcagctgctgttcttgcagtttctgcacgcgccagcgcctggattatcggcattcaatccgcccaaattaaggcgattgaaaacgaccaccactggcacgaaggcaactactacgaatccggctgcaacccagccaccggactcggcgccgcccgacgcatcgcccacctcacctaccgtggcgaactagaaatcgacgaacgcttcggcaccaaagcccaaaagaacgaaaacccactcggtccctaccgcaagcccgaccagcgcttcgccgtggaatcctacttggactaccaagcagacaagctagtacagcgtttcgacgccggctcctacgtcttgctcaccgacgccctcaaccgccacgacattggtcgcgaccgcggaggcctcaacaaggcactcgaatccatcaaagttccagtccttgtcgcaggcgtagataccgatattcggtacccctaccaccagcaagaacacctctccagaaacctgggaaatctactggcaatggcaaaaatcgtatcccctgtcggccacgatgctttcctcaccgaaagccgccaaatggatcgcatcgtgaggaacttcttcagcctcatctccccagacgaagacaacccttcgacctacatcgagttctacatctaa

SEQ ID NO: 81 - protein, 377 aa, Artificial Sequence
  Q176T,L313R
MPTLAPSGQLEIQAIGDVSTEAGAIITNAEIAYHRWGEYRVDKEGRSNVVLIEHALTGDSNAADWWADLLGPGKAINTDIYCVICTNVIGGCNGSTGPGSMHPDGNFWGNRFPATSIRDQVNAEKQFLDALGITTVAAVLGGSMGGARTLEWAAMYPETVGAAAVLAVSARASAWTIGIQSAQIKAIENDHHWHEGNYYESGCNPATGLGAARRIAHLTYRGELEIDERFGTKAQKNENPLGPYRKPDQRFAVESYLDYQADKLVQRFDAGSYVLLTDALNRHDIGRDRGGLNKALESIKVPVLVAGVDTDIRYPYHQQEHLSRNLGNLLAMAKIVSPVGHDAFLTESRQMDRIVRNFFSLISPDEDNPSTYIEFYI

SEQ ID NO: 82 - DNA, 1134 bp, Artificial Sequence
  Q176T,L313R
atgcccaccctcgcgccttcaggtcaacttgaaatccaagcgatcggtgatgtctccaccgaagccggagcaatcattacaaacgctgaaatcgcctatcaccgctggggtgaataccgcgtagataaagaaggacgcagcaatgtcgttctcatcgaacacgccctcactggagattccaacgcagccgattggtgggctgacttgctcggtcccggcaaagccatcaacactgatatttactgcgtgatctgtaccaacgtcatcggtggttgcaacggttccaccggacctggctccatgcatccagatggaaatttctggggtaatcgcttccccgccacgtccattcgtgatcaggtaaacgccgaaaaacaattcctcgacgcactcggcatcaccacggtcgccgcagtacttggtggttccatgggtggtgcccgcaccctagagtgggccgcaatgtacccagaaactgttggcgcagctgctgttcttgcagtttctgcacgcgccagcgcctggactatcggcattcaatccgcccaaattaaggcgattgaaaacgaccaccactggcacgaaggcaactactacgaatccggctgcaacccagccaccggactcggcgccgcccgacgcatcgcccacctcacctaccgtggcgaactagaaatcgacgaacgcttcggcaccaaagcccaaaagaacgaaaacccactcggtccctaccgcaagcccgaccagcgcttcgccgtggaatcctacttggactaccaagcagacaagctagtacagcgtttcgacgccggctcctacgtcttgctcaccgacgccctcaaccgccacgacattggtcgcgaccgcggaggcctcaacaaggcactcgaatccatcaaagttccagtccttgtcgcaggcgtagataccgatattcggtacccctaccaccagcaagaacacctctccagaaacctgggaaatctactggcaatggcaaaaatcgtatcccctgtcggccacgatgctttcctcaccgaaagccgccaaatggatcgcatcgtgaggaacttcttcagcctcatctccccagacgaagacaacccttcgacctacatcgagttctacatctaa

SEQ ID NO: 83 - protein, 377 aa, Artificial Sequence
  Q176R,L313R
MPTLAPSGQLEIQAIGDVSTEAGAIITNAEIAYHRWGEYRVDKEGRSNVVLIEHALTGDSNAADWWADLLGPGKAINTDIYCVICTNVIGGCNGSTGPGSMHPDGNFWGNRFPATSIRDQVNAEKQFLDALGITTVAAVLGGSMGGARTLEWAAMYPETVGAAAVLAVSARASAWRIGIQSAQIKAIENDHHWHEGNYYESGCNPATGLGAARRIAHLTYRGELEIDERFGTKAQKNENPLGPYRKPDQRFAVESYLDYQADKLVQRFDAGSYVLLTDALNRHDIGRDRGGLNKALESIKVPVLVAGVDTDIRYPYHQQEHLSRNLGNLLAMAKIVSPVGHDAFLTESRQMDRIVRNFFSLISPDEDNPSTYIEFYI

SEQ ID NO: 84 - DNA, 1134 bp, Artificial Sequence
  Q176R,L313R
atgcccaccctcgcgccttcaggtcaacttgaaatccaagcgatcggtgatgtctccaccgaagccggagcaatcattacaaacgctgaaatcgcctatcaccgctggggtgaataccgcgtagataaagaaggacgcagcaatgtcgttctcatcgaacacgccctcactggagattccaacgcagccgattggtgggctgacttgctcggtcccggcaaagccatcaacactgatatttactgcgtgatctgtaccaacgtcatcggtggttgcaacggttccaccggacctggctccatgcatccagatggaaatttctggggtaatcgcttccccgccacgtccattcgtgatcaggtaaacgccgaaaaacaattcctcgacgcactcggcatcaccacggtcgccgcagtacttggtggttccatgggtggtgcccgcaccctagagtgggccgcaatgtacccagaaactgttggcgcagctgctgttcttgcagtttctgcacgcgccagcgcctggcgcatcggcattcaatccgcccaaattaaggcgattgaaaacgaccaccactggcacgaaggcaactactacgaatccggctgcaacccagccaccggactcggcgccgcccgacgcatcgcccacctcacctaccgtggcgaactagaaatcgacgaacgcttcggcaccaaagcccaaaagaacgaaaacccactcggtccctaccgcaagcccgaccagcgcttcgccgtggaatcctacttggactaccaagcagacaagctagtacagcgtttcgacgccggctcctacgtcttgctcaccgacgccctcaaccgccacgacattggtcgcgaccgcggaggcctcaacaaggcactcgaatccatcaaagttccagtccttgtcgcaggcgtagataccgatattcggtacccctaccaccagcaagaacacctctccagaaacctgggaaatctactggcaatggcaaaaatcgtatcccctgtcggccacgatgctttcctcaccgaaagccgccaaatggatcgcatcgtgaggaacttcttcagcctcatctccccagacgaagacaacccttcgacctacatcgagttctacatctaa

SEQ ID NO: 85 - protein, 377 aa, Artificial Sequence
  Q176K,L313R
MPTLAPSGQLEIQAIGDVSTEAGAIITNAEIAYHRWGEYRVDKEGRSNVVLIEHALTGDSNAADWWADLLGPGKAINTDIYCVICTNVIGGCNGSTGPGSMHPDGNFWGNRFPATSIRDQVNAEKQFLDALGITTVAAVLGGSMGGARTLEWAAMYPETVGAAAVLAVSARASAWKIGIQSAQIKAIENDHHWHEGNYYESGCNPATGLGAARRIAHLTYRGELEIDERFGTKAQKNENPLGPYRKPDQRFAVESYLDYQADKLVQRFDAGSYVLLTDALNRHDIGRDRGGLNKALESIKVPVLVAGVDTDIRYPYHQQEHLSRNLGNLLAMAKIVSPVGHDAFLTESRQMDRIVRNFFSLISPDEDNPSTYIEFYI

SEQ ID NO: 86 - DNA, 1134 bp, Artificial Sequence
  Q176K,L313R
atgcccaccctcgcgccttcaggtcaacttgaaatccaagcgatcggtgatgtctccaccgaagccggagcaatcattacaaacgctgaaatcgcctatcaccgctggggtgaataccgcgtagataaagaaggacgcagcaatgtcgttctcatcgaacacgccctcactggagattccaacgcagccgattggtgggctgacttgctcggtcccggcaaagccatcaacactgatatttactgcgtgatctgtaccaacgtcatcggtggttgcaacggttccaccggacctggctccatgcatccagatggaaatttctggggtaatcgcttccccgccacgtccattcgtgatcaggtaaacgccgaaaaacaattcctcgacgcactcggcatcaccacggtcgccgcagtacttggtggttccatgggtggtgcccgcaccctagagtgggccgcaatgtacccagaaactgttggcgcagctgctgttcttgcagtttctgcacgcgccagcgcctggaaaatcggcattcaatccgcccaaattaaggcgattgaaaacgaccaccactggcacgaaggcaactactacgaatccggctgcaacccagccaccggactcggcgccgcccgacgcatcgcccacctcacctaccgtggcgaactagaaatcgacgaacgcttcggcaccaaagcccaaaagaacgaaaacccactcggtccctaccgcaagcccgaccagcgcttcgccgtggaatcctacttggactaccaagcagacaagctagtacagcgtttcgacgccggctcctacgtcttgctcaccgacgccctcaaccgccacgacattggtcgcgaccgcggaggcctcaacaaggcactcgaatccatcaaagttccagtccttgtcgcaggcgtagataccgatattcggtacccctaccaccagcaagaacacctctccagaaacctgggaaatctactggcaatggcaaaaatcgtatcccctgtcggccacgatgctttcctcaccgaaagccgccaaatggatcgcatcgtgaggaacttcttcagcctcatctccccagacgaagacaacccttcgacctacatcgagttctacatctaa

SEQ ID NO: 87 - protein, 377 aa, Artificial Sequence
  Q176V,L313R
MPTLAPSGQLEIQAIGDVSTEAGAIITNAEIAYHRWGEYRVDKEGRSNVVLIEHALTGDSNAADWWADLLGPGKAINTDIYCVICTNVIGGCNGSTGPGSMHPDGNFWGNRFPATSIRDQVNAEKQFLDALGITTVAAVLGGSMGGARTLEWAAMYPETVGAAAVLAVSARASAWVIGIQSAQIKAIENDHHWHEGNYYESGCNPATGLGAARRIAHLTYRGELEIDERFGTKAQKNENPLGPYRKPDQRFAVESYLDYQADKLVQRFDAGSYVLLTDALNRHDIGRDRGGLNKALESIKVPVLVAGVDTDIRYPYHQQEHLSRNLGNLLAMAKIVSPVGHDAFLTESRQMDRIVRNFFSLISPDEDNPSTYIEFYI

SEQ ID NO: 88 - DNA, 1134 bp, Artificial Sequence
  Q176V,L313R
atgcccaccctcgcgccttcaggtcaacttgaaatccaagcgatcggtgatgtctccaccgaagccggagcaatcattacaaacgctgaaatcgcctatcaccgctggggtgaataccgcgtagataaagaaggacgcagcaatgtcgttctcatcgaacacgccctcactggagattccaacgcagccgattggtgggctgacttgctcggtcccggcaaagccatcaacactgatatttactgcgtgatctgtaccaacgtcatcggtggttgcaacggttccaccggacctggctccatgcatccagatggaaatttctggggtaatcgcttccccgccacgtccattcgtgatcaggtaaacgccgaaaaacaattcctcgacgcactcggcatcaccacggtcgccgcagtacttggtggttccatgggtggtgcccgcaccctagagtgggccgcaatgtacccagaaactgttggcgcagctgctgttcttgcagtttctgcacgcgccagcgcctgggttatcggcattcaatccgcccaaattaaggcgattgaaaacgaccaccactggcacgaaggcaactactacgaatccggctgcaacccagccaccggactcggcgccgcccgacgcatcgcccacctcacctaccgtggcgaactagaaatcgacgaacgcttcggcaccaaagcccaaaagaacgaaaacccactcggtccctaccgcaagcccgaccagcgcttcgccgtggaatcctacttggactaccaagcagacaagctagtacagcgtttcgacgccggctcctacgtcttgctcaccgacgccctcaaccgccacgacattggtcgcgaccgcggaggcctcaacaaggcactcgaatccatcaaagttccagtccttgtcgcaggcgtagataccgatattcggtacccctaccaccagcaagaacacctctccagaaacctgggaaatctactggcaatggcaaaaatcgtatcccctgtcggccacgatgctttcctcaccgaaagccgccaaatggatcgcatcgtgaggaacttcttcagcctcatctccccagacgaagacaacccttcgacctacatcgagttctacatctaa

SEQ ID NO: 89 - protein, 377 aa, Artificial Sequence
  Q176A,L313R
MPTLAPSGQLEIQAIGDVSTEAGAIITNAEIAYHRWGEYRVDKEGRSNVVLIEHALTGDSNAADWWADLLGPGKAINTDIYCVICTNVIGGCNGSTGPGSMHPDGNFWGNRFPATSIRDQVNAEKQFLDALGITTVAAVLGGSMGGARTLEWAAMYPETVGAAAVLAVSARASAWAIGIQSAQIKAIENDHHWHEGNYYESGCNPATGLGAARRIAHLTYRGELEIDERFGTKAQKNENPLGPYRKPDQRFAVESYLDYQADKLVQRFDAGSYVLLTDALNRHDIGRDRGGLNKALESIKVPVLVAGVDTDIRYPYHQQEHLSRNLGNLLAMAKIVSPVGHDAFLTESRQMDRIVRNFFSLISPDEDNPSTYIEFYI

SEQ ID NO: 90 - DNA, 1134 bp, Artificial Sequence
  Q176A,L313R
atgcccaccctcgcgccttcaggtcaacttgaaatccaagcgatcggtgatgtctccaccgaagccggagcaatcattacaaacgctgaaatcgcctatcaccgctggggtgaataccgcgtagataaagaaggacgcagcaatgtcgttctcatcgaacacgccctcactggagattccaacgcagccgattggtgggctgacttgctcggtcccggcaaagccatcaacactgatatttactgcgtgatctgtaccaacgtcatcggtggttgcaacggttccaccggacctggctccatgcatccagatggaaatttctggggtaatcgcttccccgccacgtccattcgtgatcaggtaaacgccgaaaaacaattcctcgacgcactcggcatcaccacggtcgccgcagtacttggtggttccatgggtggtgcccgcaccctagagtgggccgcaatgtacccagaaactgttggcgcagctgctgttcttgcagtttctgcacgcgccagcgcctgggcaatcggcattcaatccgcccaaattaaggcgattgaaaacgaccaccactggcacgaaggcaactactacgaatccggctgcaacccagccaccggactcggcgccgcccgacgcatcgcccacctcacctaccgtggcgaactagaaatcgacgaacgcttcggcaccaaagcccaaaagaacgaaaacccactcggtccctaccgcaagcccgaccagcgcttcgccgtggaatcctacttggactaccaagcagacaagctagtacagcgtttcgacgccggctcctacgtcttgctcaccgacgccctcaaccgccacgacattggtcgcgaccgcggaggcctcaacaaggcactcgaatccatcaaagttccagtccttgtcgcaggcgtagataccgatattcggtacccctaccaccagcaagaacacctctccagaaacctgggaaatctactggcaatggcaaaaatcgtatcccctgtcggccacgatgctttcctcaccgaaagccgccaaatggatcgcatcgtgaggaacttcttcagcctcatctccccagacgaagacaacccttcgacctacatcgagttctacatctaa

SEQ ID NO: 91 - protein, 377 aa, Artificial Sequence
  Q176D,L313R
MPTLAPSGQLEIQAIGDVSTEAGAIITNAEIAYHRWGEYRVDKEGRSNVVLIEHALTGDSNAADWWADLLGPGKAINTDIYCVICTNVIGGCNGSTGPGSMHPDGNFWGNRFPATSIRDQVNAEKQFLDALGITTVAAVLGGSMGGARTLEWAAMYPETVGAAAVLAVSARASAWDIGIQSAQIKAIENDHHWHEGNYYESGCNPATGLGAARRIAHLTYRGELEIDERFGTKAQKNENPLGPYRKPDQRFAVESYLDYQADKLVQRFDAGSYVLLTDALNRHDIGRDRGGLNKALESIKVPVLVAGVDTDIRYPYHQQEHLSRNLGNLLAMAKIVSPVGHDAFLTESRQMDRIVRNFFSLISPDEDNPSTYIEFYI

SEQ ID NO: 92 - DNA, 1134 bp, Artificial Sequence
  Q176D,L313R
atgcccaccctcgcgccttcaggtcaacttgaaatccaagcgatcggtgatgtctccaccgaagccggagcaatcattacaaacgctgaaatcgcctatcaccgctggggtgaataccgcgtagataaagaaggacgcagcaatgtcgttctcatcgaacacgccctcactggagattccaacgcagccgattggtgggctgacttgctcggtcccggcaaagccatcaacactgatatttactgcgtgatctgtaccaacgtcatcggtggttgcaacggttccaccggacctggctccatgcatccagatggaaatttctggggtaatcgcttccccgccacgtccattcgtgatcaggtaaacgccgaaaaacaattcctcgacgcactcggcatcaccacggtcgccgcagtacttggtggttccatgggtggtgcccgcaccctagagtgggccgcaatgtacccagaaactgttggcgcagctgctgttcttgcagtttctgcacgcgccagcgcctgggacatcggcattcaatccgcccaaattaaggcgattgaaaacgaccaccactggcacgaaggcaactactacgaatccggctgcaacccagccaccggactcggcgccgcccgacgcatcgcccacctcacctaccgtggcgaactagaaatcgacgaacgcttcggcaccaaagcccaaaagaacgaaaacccactcggtccctaccgcaagcccgaccagcgcttcgccgtggaatcctacttggactaccaagcagacaagctagtacagcgtttcgacgccggctcctacgtcttgctcaccgacgccctcaaccgccacgacattggtcgcgaccgcggaggcctcaacaaggcactcgaatccatcaaagttccagtccttgtcgcaggcgtagataccgatattcggtacccctaccaccagcaagaacacctctccagaaacctgggaaatctactggcaatggcaaaaatcgtatcccctgtcggccacgatgctttcctcaccgaaagccgccaaatggatcgcatcgtgaggaacttcttcagcctcatctccccagacgaagacaacccttcgacctacatcgagttctacatctaa

SEQ ID NO: 93 - protein, 377 aa, Artificial Sequence
  Q176E,L313R
MPTLAPSGQLEIQAIGDVSTEAGAIITNAEIAYHRWGEYRVDKEGRSNVVLIEHALTGDSNAADWWADLLGPGKAINTDIYCVICTNVIGGCNGSTGPGSMHPDGNFWGNRFPATSIRDQVNAEKQFLDALGITTVAAVLGGSMGGARTLEWAAMYPETVGAAAVLAVSARASAWEIGIQSAQIKAIENDHHWHEGNYYESGCNPATGLGAARRIAHLTYRGELEIDERFGTKAQKNENPLGPYRKPDQRFAVESYLDYQADKLVQRFDAGSYVLLTDALNRHDIGRDRGGLNKALESIKVPVLVAGVDTDIRYPYHQQEHLSRNLGNLLAMAKIVSPVGHDAFLTESRQMDRIVRNFFSLISPDEDNPSTYIEFYI

SEQ ID NO: 94 - DNA, 1134 bp, Artificial Sequence
  Q176E,L313R
atgcccaccctcgcgccttcaggtcaacttgaaatccaagcgatcggtgatgtctccaccgaagccggagcaatcattacaaacgctgaaatcgcctatcaccgctggggtgaataccgcgtagataaagaaggacgcagcaatgtcgttctcatcgaacacgccctcactggagattccaacgcagccgattggtgggctgacttgctcggtcccggcaaagccatcaacactgatatttactgcgtgatctgtaccaacgtcatcggtggttgcaacggttccaccggacctggctccatgcatccagatggaaatttctggggtaatcgcttccccgccacgtccattcgtgatcaggtaaacgccgaaaaacaattcctcgacgcactcggcatcaccacggtcgccgcagtacttggtggttccatgggtggtgcccgcaccctagagtgggccgcaatgtacccagaaactgttggcgcagctgctgttcttgcagtttctgcacgcgccagcgcctgggagatcggcattcaatccgcccaaattaaggcgattgaaaacgaccaccactggcacgaaggcaactactacgaatccggctgcaacccagccaccggactcggcgccgcccgacgcatcgcccacctcacctaccgtggcgaactagaaatcgacgaacgcttcggcaccaaagcccaaaagaacgaaaacccactcggtccctaccgcaagcccgaccagcgcttcgccgtggaatcctacttggactaccaagcagacaagctagtacagcgtttcgacgccggctcctacgtcttgctcaccgacgccctcaaccgccacgacattggtcgcgaccgcggaggcctcaacaaggcactcgaatccatcaaagttccagtccttgtcgcaggcgtagataccgatattcggtacccctaccaccagcaagaacacctctccagaaacctgggaaatctactggcaatggcaaaaatcgtatcccctgtcggccacgatgctttcctcaccgaaagccgccaaatggatcgcatcgtgaggaacttcttcagcctcatctccccagacgaagacaacccttcgacctacatcgagttctacatctaa

SEQ ID NO: 95 - protein, 377 aa, Artificial Sequence
  Q176G,L313R
MPTLAPSGQLEIQAIGDVSTEAGAIITNAEIAYHRWGEYRVDKEGRSNVVLIEHALTGDSNAADWWADLLGPGKAINTDIYCVICTNVIGGCNGSTGPGSMHPDGNFWGNRFPATSIRDQVNAEKQFLDALGITTVAAVLGGSMGGARTLEWAAMYPETVGAAAVLAVSARASAWGIGIQSAQIKAIENDHHWHEGNYYESGCNPATGLGAARRIAHLTYRGELEIDERFGTKAQKNENPLGPYRKPDQRFAVESYLDYQADKLVQRFDAGSYVLLTDALNRHDIGRDRGGLNKALESIKVPVLVAGVDTDIRYPYHQQEHLSRNLGNLLAMAKIVSPVGHDAFLTESRQMDRIVRNFFSLISPDEDNPSTYIEFYI

SEQ ID NO: 96 - DNA, 1134 bp, Artificial Sequence
  Q176G,L313R
atgcccaccctcgcgccttcaggtcaacttgaaatccaagcgatcggtgatgtctccaccgaagccggagcaatcattacaaacgctgaaatcgcctatcaccgctggggtgaataccgcgtagataaagaaggacgcagcaatgtcgttctcatcgaacacgccctcactggagattccaacgcagccgattggtgggctgacttgctcggtcccggcaaagccatcaacactgatatttactgcgtgatctgtaccaacgtcatcggtggttgcaacggttccaccggacctggctccatgcatccagatggaaatttctggggtaatcgcttccccgccacgtccattcgtgatcaggtaaacgccgaaaaacaattcctcgacgcactcggcatcaccacggtcgccgcagtacttggtggttccatgggtggtgcccgcaccctagagtgggccgcaatgtacccagaaactgttggcgcagctgctgttcttgcagtttctgcacgcgccagcgcctggggcatcggcattcaatccgcccaaattaaggcgattgaaaacgaccaccactggcacgaaggcaactactacgaatccggctgcaacccagccaccggactcggcgccgcccgacgcatcgcccacctcacctaccgtggcgaactagaaatcgacgaacgcttcggcaccaaagcccaaaagaacgaaaacccactcggtccctaccgcaagcccgaccagcgcttcgccgtggaatcctacttggactaccaagcagacaagctagtacagcgtttcgacgccggctcctacgtcttgctcaccgacgccctcaaccgccacgacattggtcgcgaccgcggaggcctcaacaaggcactcgaatccatcaaagttccagtccttgtcgcaggcgtagataccgatattcggtacccctaccaccagcaagaacacctctccagaaacctgggaaatctactggcaatggcaaaaatcgtatcccctgtcggccacgatgctttcctcaccgaaagccgccaaatggatcgcatcgtgaggaacttcttcagcctcatctccccagacgaagacaacccttcgacctacatcgagttctacatctaa

SEQ ID NO: 97 - protein, 377 aa, Artificial Sequence
  Q176W,L313R
MPTLAPSGQLEIQAIGDVSTEAGAIITNAEIAYHRWGEYRVDKEGRSNVVLIEHALTGDSNAADWWADLLGPGKAINTDIYCVICTNVIGGCNGSTGPGSMHPDGNFWGNRFPATSIRDQVNAEKQFLDALGITTVAAVLGGSMGGARTLEWAAMYPETVGAAAVLAVSARASAWWIGIQSAQIKAIENDHHWHEGNYYESGCNPATGLGAARRIAHLTYRGELEIDERFGTKAQKNENPLGPYRKPDQRFAVESYLDYQADKLVQRFDAGSYVLLTDALNRHDIGRDRGGLNKALESIKVPVLVAGVDTDIRYPYHQQEHLSRNLGNLLAMAKIVSPVGHDAFLTESRQMDRIVRNFFSLISPDEDNPSTYIEFYI

SEQ ID NO: 98 - DNA, 1134 bp, Artificial Sequence
  Q176W,L313R
atgcccaccctcgcgccttcaggtcaacttgaaatccaagcgatcggtgatgtctccaccgaagccggagcaatcattacaaacgctgaaatcgcctatcaccgctggggtgaataccgcgtagataaagaaggacgcagcaatgtcgttctcatcgaacacgccctcactggagattccaacgcagccgattggtgggctgacttgctcggtcccggcaaagccatcaacactgatatttactgcgtgatctgtaccaacgtcatcggtggttgcaacggttccaccggacctggctccatgcatccagatggaaatttctggggtaatcgcttccccgccacgtccattcgtgatcaggtaaacgccgaaaaacaattcctcgacgcactcggcatcaccacggtcgccgcagtacttggtggttccatgggtggtgcccgcaccctagagtgggccgcaatgtacccagaaactgttggcgcagctgctgttcttgcagtttctgcacgcgccagcgcctggtggatcggcattcaatccgcccaaattaaggcgattgaaaacgaccaccactggcacgaaggcaactactacgaatccggctgcaacccagccaccggactcggcgccgcccgacgcatcgcccacctcacctaccgtggcgaactagaaatcgacgaacgcttcggcaccaaagcccaaaagaacgaaaacccactcggtccctaccgcaagcccgaccagcgcttcgccgtggaatcctacttggactaccaagcagacaagctagtacagcgtttcgacgccggctcctacgtcttgctcaccgacgccctcaaccgccacgacattggtcgcgaccgcggaggcctcaacaaggcactcgaatccatcaaagttccagtccttgtcgcaggcgtagataccgatattcggtacccctaccaccagcaagaacacctctccagaaacctgggaaatctactggcaatggcaaaaatcgtatcccctgtcggccacgatgctttcctcaccgaaagccgccaaatggatcgcatcgtgaggaacttcttcagcctcatctccccagacgaagacaacccttcgacctacatcgagttctacatctaa